European Patent Application EP 4 115 740 A1, published January 11, 2023. Title: MUTANT TRANSGLUTAMINASE. Applicant: Ajinomoto Co., Inc. The sequence listing filed with the application follows.

SEQUENCE LISTING (24 sequences)

SEQ ID NO: 1 - DNA, 996 bp, Streptoverticillium mobaraense
gactccgacgacagggtcacccctcccgccgagccgctcgacaggatgcccgacccgtaccgtccctcgtacggcagggccgagacggtcgtcaacaactacatacgcaagtggcagcaggtctacagccaccgcgacggcaggaagcagcagatgaccgaggagcagcgggagtggctgtcctacggctgcgtcggtgtcacctgggtcaattcgggtcagtacccgacgaacagactggccttcgcgtccttcgacgaggacaggttcaagaacgagctgaagaacggcaggccccggtccggcgagacgcgggcggagttcgagggccgcgtcgcgaaggagagcttcgacgaggagaagggcttccagcgggcgcgtgaggtggcgtccgtcatgaacagggccctggagaacgcccacgacgagagcgcttacctcgacaacctcaagaaggaactggcgaacggcaacgacgccctgcgcaacgaggacgcccgttccccgttctactcggcgctgcggaacacgccgtccttcaaggagcggaacggaggcaatcacgacccgtccaggatgaaggccgtcatctactcgaagcacttctggagcggccaggaccggtcgagttcggccgacaagaggaagtacggcgacccggacgccttccgccccgccccgggcaccggcctggtcgacatgtcgagggacaggaacattccgcgcagccccaccagccccggtgagggattcgtcaatttcgactacggctggttcggcgcccagacggaagcggacgccgacaagaccgtctggacccacggaaatcactatcacgcgcccaatggcagcctgggtgccatgcatgtctacgagagcaagttccgcaactggtccgagggttactcggacttcgaccgcggagcctatgtgatcaccttcatccccaagagctggaacaccgcccccgacaaggtaaagcagggctggccgtga

SEQ ID NO: 2 - protein, 331 aa, Streptoverticillium mobaraense
DSDDRVTPPAEPLDRMPDPYRPSYGRAETVVNNYIRKWQQVYSHRDGRKQQMTEEQREWLSYGCVGVTWVNSGQYPTNRLAFASFDEDRFKNELKNGRPRSGETRAEFEGRVAKESFDEEKGFQRAREVASVMNRALENAHDESAYLDNLKKELANGNDALRNEDARSPFYSALRNTPSFKERNGGNHDPSRMKAVIYSKHFWSGQDRSSSADKRKYGDPDAFRPAPGTGLVDMSRDRNIPRSPTSPGEGFVNFDYGWFGAQTEADADKTVWTHGNHYHAPNGSLGAMHVYESKFRNWSEGYSDFDRGAYVITFIPKSWNTAPDKVKQGWP

SEQ ID NO: 3 - DNA, 1131 bp, Streptoverticillium mobaraense
gacaatggcgcgggggaagagacgaagtcctacgccgaaacctaccgcctcacggcggatgacgtcgcgaacatcaacgcgctcaacgaaagcgctccggccgcttcgagcgccggcccgtcgttccgggcccccgactccgacgacagggtcacccctcccgccgagccgctcgacaggatgcccgacccgtaccgtccctcgtacggcagggccgagacggtcgtcaacaactacatacgcaagtggcagcaggtctacagccaccgcgacggcaggaagcagcagatgaccgaggagcagcgggagtggctgtcctacggctgcgtcggtgtcacctgggtcaattcgggtcagtacccgacgaacagactggccttcgcgtccttcgacgaggacaggttcaagaacgagctgaagaacggcaggccccggtccggcgagacgcgggcggagttcgagggccgcgtcgcgaaggagagcttcgacgaggagaagggcttccagcgggcgcgtgaggtggcgtccgtcatgaacagggccctggagaacgcccacgacgagagcgcttacctcgacaacctcaagaaggaactggcgaacggcaacgacgccctgcgcaacgaggacgcccgttccccgttctactcggcgctgcggaacacgccgtccttcaaggagcggaacggaggcaatcacgacccgtccaggatgaaggccgtcatctactcgaagcacttctggagcggccaggaccggtcgagttcggccgacaagaggaagtacggcgacccggacgccttccgccccgccccgggcaccggcctggtcgacatgtcgagggacaggaacattccgcgcagccccaccagccccggtgagggattcgtcaatttcgactacggctggttcggcgcccagacggaagcggacgccgacaagaccgtctggacccacggaaatcactatcacgcgcccaatggcagcctgggtgccatgcatgtctacgagagcaagttccgcaactggtccgagggttactcggacttcgaccgcggagcctatgtgatcaccttcatccccaagagctggaacaccgcccccgacaaggtaaagcagggctggccgtga

SEQ ID NO: 4 - protein, 376 aa, Streptoverticillium mobaraense
DNGAGEETKSYAETYRLTADDVANINALNESAPAASSAGPSFRAPDSDDRVTPPAEPLDRMPDPYRPSYGRAETVVNNYIRKWQQVYSHRDGRKQQMTEEQREWLSYGCVGVTWVNSGQYPTNRLAFASFDEDRFKNELKNGRPRSGETRAEFEGRVAKESFDEEKGFQRAREVASVMNRALENAHDESAYLDNLKKELANGNDALRNEDARSPFYSALRNTPSFKERNGGNHDPSRMKAVIYSKHFWSGQDRSSSADKRKYGDPDAFRPAPGTGLVDMSRDRNIPRSPTSPGEGFVNFDYGWFGAQTEADADKTVWTHGNHYHAPNGSLGAMHVYESKFRNWSEGYSDFDRGAYVITFIPKSWNTAPDKVKQGWP

SEQ ID NO: 5 - DNA, 21 bp, Artificial Sequence
  primer
acaaggactgctcccaaagat

SEQ ID NO: 6 - DNA, 21 bp, Artificial Sequence
  primer
gggagcagtccttgtcgcgtt

SEQ ID NO: 7 - DNA, 28 bp, Artificial Sequence
  primer
gtcgggcgtcctgtcgagcggctcggcg

SEQ ID NO: 8 - DNA, 28 bp, Artificial Sequence
  primer
gacaggacgcccgacccgtaccgtccct

SEQ ID NO: 9 - DNA, 28 bp, Artificial Sequence
  primer
gcgtatgaagttgttgacgaccgtctcg

SEQ ID NO: 10 - DNA, 28 bp, Artificial Sequence
  primer
aacaacttcatacgcaagtggcagcagg

SEQ ID NO: 11 - DNA, 28 bp, Artificial Sequence
  primer
ctgctgaaacttgcgtatgtagttgttg

SEQ ID NO: 12 - DNA, 29 bp, Artificial Sequence
  primer
cgcaagtttcagcaggtctacagccaccg

SEQ ID NO: 13 - DNA, 28 bp, Artificial Sequence
  primer
ctgccggggcggtggctgtagacctgct

SEQ ID NO: 14 - DNA, 29 bp, Artificial Sequence
  primer
ccaccgccccggcaggaagcagcagatga

SEQ ID NO: 15 - DNA, 28 bp, Artificial Sequence
  primer
tgcttcgcgtagatgacggccttcatcc

SEQ ID NO: 16 - DNA, 28 bp, Artificial Sequence
  primer
catctacgcgaagcacttctggagcggc

SEQ ID NO: 17 - DNA, 28 bp, Artificial Sequence
  primer
gtctggcagccgaaccagccgtagtcga

SEQ ID NO: 18 - DNA, 29 bp, Artificial Sequence
  primer
gttcggctgccagacggaagcggacgccg

SEQ ID NO: 19 - DNA, 29 bp, Artificial Sequence
  primer
ggtccagcaggtcttgtcggcgtccgctt

SEQ ID NO: 20 - DNA, 28 bp, Artificial Sequence
  primer
aagacctgctggacccacggaaatcact

SEQ ID NO: 21 - DNA, 28 bp, Artificial Sequence
  primer
tcggggcaggtgttccagctcttgggga

SEQ ID NO: 22 - DNA, 29 bp, Artificial Sequence
  primer
gaacacctgccccgacaaggtaaagcagg

SEQ ID NO: 23 - DNA, 29 bp, Artificial Sequence
  primer
ctgcttgcacttgtcgggggcggtgttcc

SEQ ID NO: 24 - DNA, 29 bp, Artificial Sequence
  primer
gacaagtgcaagcagggctggccgtgatg